European Patent Specification EP 3 332 034 B1, published September 25, 2024. Title: SYSTEMS AND METHODS FOR GENOMIC ANALYSIS. Applicant: Arc Bio, LLC Watson, Thomas J Quiroz-Zarate, Alejandro van Aggelen, Helen Olivares-Amaya, Roberto Coronado Sroka, Eduardo Angulo Sermeno, Carlos Fimbres Jurado, Fernando Garcia-Inda, Abraham Fontove Herrera, Fernando. The sequence listing filed with the application follows.

SEQUENCE LISTING (12 sequences)

SEQ ID NO: 1 - DNA, 10 bp, Artificial Sequence
  synthetic
acttaactgg

SEQ ID NO: 2 - DNA, 45 bp, Artificial Sequence
  synthetic
agcatgttagataagatagctgtgctagtaggcagtcagcgccat

SEQ ID NO: 3 - DNA, 17 bp, Artificial Sequence
  synthetic
ttagataaaggatactg

SEQ ID NO: 4 - DNA, 14 bp, Artificial Sequence
  synthetic
aaaagataaggata

SEQ ID NO: 5 - DNA, 11 bp, Artificial Sequence
  synthetic
gcctaagctaa

SEQ ID NO: 6 - DNA, 17 bp, Artificial Sequence
  synthetic
ttagataaaggatactg

SEQ ID NO: 7 - DNA, 14 bp, Artificial Sequence
  synthetic
aaaagataaggata

SEQ ID NO: 8 - DNA, 11 bp, Artificial Sequence
  synthetic
gcctaagctaa

SEQ ID NO: 9 - DNA, 11 bp, Artificial Sequence
  synthetic
atagcttcagc

SEQ ID NO: 10 - DNA, 11 bp, Artificial Sequence
  synthetic
gctgcttaggc

SEQ ID NO: 11 - DNA, 11 bp, Artificial Sequence
  synthetic
aatgaacaatg

SEQ ID NO: 12 - DNA, 21 bp, Artificial Sequence
  synthetic
ggggcaggtaatgaacgacgg